European Patent Application EP 4 509 522 A1, published February 19, 2025. Title: A TGFbeta switch receptor, a nucleic acid encoding it, cells and pharmaceutical compositions comprising the same. Applicant: Max-Delbrueck-Centrum fuer Molekulare Medizin in der Helmholtz-Gemeinschaft. The sequence listing filed with the application follows.

SEQUENCE LISTING (56 sequences)

SEQ ID NO: 1 - protein, 5 aa, synthetic construct
  source 1..5: note = HCDR1 / PET1073G12
SNVIS

SEQ ID NO: 2 - protein, 17 aa, synthetic construct
  source 1..17: note = HCDR2 / PET1073G12
GVIPIVDIANYAQRFKG

SEQ ID NO: 3 - protein, 11 aa, synthetic construct
  source 1..11: note = HCDR3 / PET1073G12
TLGLVLDAMDY

SEQ ID NO: 4 - protein, 12 aa, synthetic construct
  source 1..12: note = VCDR1 / PET1073G12
RASQSLGSSYLA

SEQ ID NO: 5 - protein, 7 aa, synthetic construct
  source 1..7: note = VCDR2 / PET1073G12
GASSRAP

SEQ ID NO: 6 - protein, 9 aa, synthetic construct
  source 1..9: note = VCDR3/ PET1073G12
QQYADSPIT

SEQ ID NO: 7 - protein, 120 aa, synthetic construct
  source 1..120: note = Heavy chain variable domain / PET1073G12
QVQLVQSGAEVKKPGSSVKVSCKASGYTPSSNVISWVRQAPGQGLEWMGGVIPIVDIANYAQRFKGRVTITADESTSTTYMELSSLRSEDTAVYYCASTLGLVLDAMDYWGQGTLVTVSS

SEQ ID NO: 8 - protein, 108 aa, synthetic construct
  source 1..108: note = Light chain variable domain / PET1073G12
ETVLTQSPGTLSLSPGERATLSCRASQSLGSSYLAWYQQKPGQAPRLLIYGASSRAPGIPDRFSGSGSGTDFTLTISRLEPEDFAVYYCQQYADSPITFGQGTRLEIK

SEQ ID NO: 9 - protein, 243 aa, synthetic construct
  source 1..243: note = scFv / PET1073G12
QVQLVQSGAEVKKPGSSVKVSCKASGYTPSSNVISWVRQAPGQGLEWMGGVIPIVDIANYAQRFKGRVTITADESTSTTYMELSSLRSEDTAVYYCASTLGLVLDAMDYWGQGTLVTVSSGGGGSGGGGSGGGGSETVLTQSPGTLSLSPGERATLSCRASQSLGSSYLAWYQQKPGQAPRLLIYGASSRAPGIPDRFSGSGSGTDFTLTISRLEPEDFAVYYCQQYADSPITFGQGTRLEIK

SEQ ID NO: 10 - DNA, 729 bp, synthetic construct
  source 1..729: mol_type = other DNA; note = preferred nt sequence / PET1073G12
caggtgcagctggttcaatctggcgccgaagtgaagaaacccggcagctctgtgaaggtgtcctgcaaggccagcggctacacccctagcagcaatgtgatcagctgggtccgacaggcccctggacaaggacttgaatggatgggcggcgtgatccccatcgtggatatcgccaattacgcccagcggttcaagggcagagtgaccatcacagccgatgagagcaccagcaccacctacatggaactgagcagcctgagaagcgaggacaccgccgtgtactactgtgcctctacactgggccttgtgctggacgccatggattattggggccagggcacactggtcaccgtttctagcggaggcggaggatctggtggcggaggaagtggcggaggcggttctgaaacagtgctgacacagagccccggcacactgtctcttagccctggcgaaagagccacactgagctgtagagcctctcagagcctgggcagctcttacctggcttggtatcagcagaagcccggccaggctcctagactgctgatctatggcgcctcttctagagcccctggcatccccgatagattttctggcagcggctccggcaccgacttcaccctgacaatcagcagactggaacccgaggactttgccgtgtattattgccagcagtacgccgactctcccatcacctttggccagggaacacgcctggaaatcaaa

SEQ ID NO: 11 - protein, 5 aa, synthetic construct
  source 1..5: note = HCDR1 / PET1074B9
SNVIS

SEQ ID NO: 12 - protein, 17 aa, synthetic construct
  source 1..17: note = HCDR2 / PET1074B9
GVIPIVDIANYAQRFKG

SEQ ID NO: 13 - protein, 11 aa, synthetic construct
  source 1..11: note = HCDR3 / PET1074B9
PRAFVLDAMDY

SEQ ID NO: 14 - protein, 12 aa, synthetic construct
  source 1..12: note = VCDR1 / PET1074B9
RASQSLGSSYLA

SEQ ID NO: 15 - protein, 7 aa, synthetic construct
  source 1..7: note = VCDR2 / PET1074B9
GASSRAP

SEQ ID NO: 16 - protein, 9 aa, synthetic construct
  source 1..9: note = VCDR3/ PET1074B9
QQYADSPIT

SEQ ID NO: 17 - protein, 120 aa, synthetic construct
  source 1..120: note = Heavy chain variable domain / PET1074B9
QVQLVQSGAEVKKPGSSVKVSCKASGYTFSSNVISWVRQAPGQGLEWMGGVIPIVDIANYAQRFKGRVTITADESTSTTYMELSSLRSEDTAVYYCALPRAFVLDAMDYWGQGTLVTVSS

SEQ ID NO: 18 - protein, 108 aa, synthetic construct; identical to SEQ ID NO: 8
  source 1..108: note = Light chain variable domain / PET1074B9

SEQ ID NO: 19 - protein, 243 aa, unidentified
  source 1..243: note = scFv / PET1074B9
QVQLVQSGAEVKKPGSSVKVSCKASGYTFSSNVISWVRQAPGQGLEWMGGVIPIVDIANYAQRFKGRVTITADESTSTTYMELSSLRSEDTAVYYCALPRAFVLDAMDYWGQGTLVTVSSGGGGSGGGGSGGGGSETVLTQSPGTLSLSPGERATLSCRASQSLGSSYLAWYQQKPGQAPRLLIYGASSRAPGIPDRFSGSGSGTDFTLTISRLEPEDFAVYYCQQYADSPITFGQGTRLEIK

SEQ ID NO: 20 - DNA, 729 bp, synthetic construct
  source 1..729: mol_type = other DNA; note = preferred nt sequence / PET1074B9
caggtgcagctggttcaatctggcgccgaagtgaagaaacccggcagctctgtgaaggtgtcctgcaaggccagcggctacaccttcagcagcaacgtgatcagctgggtccgacaggctcctggacaaggcttggaatggatgggcggcgtgatccccatcgtggatatcgccaattacgcccagcggttcaagggcagagtgaccatcacagccgatgagagcaccagcaccacctacatggaactgagcagcctgagaagcgaggacaccgccgtgtactattgcgccctgcctagagcctttgtgctggacgccatggattattggggccagggcacactggtcaccgtttctagcggaggcggaggatctggtggcggaggaagtggcggaggcggttctgaaacagtgctgacacagagccccggcacactgtctcttagccctggcgaaagagccacactgagctgtagagcctctcagagcctgggcagctcttacctggcttggtatcagcagaagcccggacaggcacccagactgctgatctatggcgcctcttctagagcccctggcatccccgatagattttctggcagcggctccggcaccgacttcaccctgacaatcagcagactggaacccgaggacttcgctgtgtactactgccagcagtacgccgactctcccatcacctttggccagggaacacgcctggaaatcaaa

SEQ ID NO: 21 - protein, 5 aa, synthetic construct
  source 1..5: note = HCDR1 / PET1287A10
TSFIN

SEQ ID NO: 22 - protein, 17 aa, synthetic construct
  source 1..17: note = HCDR2 / PET1287A10
GIIPIFDITNYAQKFQS

SEQ ID NO: 23 - protein, 12 aa, synthetic construct
  source 1..12: note = HCDR3 / PET1287A10
GNGNYALDAMDY

SEQ ID NO: 24 - protein, 12 aa, synthetic construct
  source 1..12: note = VCDR1 / PET1287A10
RASQSVSSSYFA

SEQ ID NO: 25 - protein, 7 aa, synthetic construct
  source 1..7: note = VCDR2 / PET1287A10
GASSRAT

SEQ ID NO: 26 - protein, 9 aa, synthetic construct
  source 1..9: note = VCDR3/ PET1287A10
QQYYDSPIT

SEQ ID NO: 27 - protein, 121 aa, synthetic construct
  source 1..121: note = Heavy chain variable domain / PET1287A10
QVQLVQSGAEVKKPGSSVKVSCKASGGTFSTSFINWVRQAPGQGLEWMGGIIPIFDITNYAQKFQSRVTITADKSTSTAYMELSSLRSEDTAVYYCARGNGNYALDAMDYWGQGTLVTVSS

SEQ ID NO: 28 - protein, 108 aa, synthetic construct
  source 1..108: note = Light chain variable domain / PET1287A10
EIVLTQSPGTLSLSPGERATLSCRASQSVSSSYFAWYQQKPGQAPRLLIYGASSRATGIPDRFSGSGSGTDFTLTISRLEPEDFAVYYCQQYYDSPITFGQGTRLEIK

SEQ ID NO: 29 - protein, 244 aa, synthetic construct
  source 1..244: note = scFv / PET1287A10
QVQLVQSGAEVKKPGSSVKVSCKASGGTFSTSFINWVRQAPGQGLEWMGGIIPIFDITNYAQKFQSRVTITADKSTSTAYMELSSLRSEDTAVYYCARGNGNYALDAMDYWGQGTLVTVSSGGGGSGGGGSGGGGSEIVLTQSPGTLSLSPGERATLSCRASQSVSSSYFAWYQQKPGQAPRLLIYGASSRATGIPDRFSGSGSGTDFTLTISRLEPEDFAVYYCQQYYDSPITFGQGTRLEIK

SEQ ID NO: 30 - DNA, 732 bp, synthetic construct
  source 1..732: mol_type = other DNA; note = preferred nt sequence / PET1287A10
caggtgcagctggttcaatctggcgccgaagtgaagaaacccggcagctctgtgaaggtgtcctgcaaagctagcggcggcaccttcagcaccagcttcatcaactgggtccgacaggcccctggacagggacttgaatggatgggcggcatcatccccatcttcgacatcaccaactacgcccagaaattccagagcagagtgaccatcaccgccgacaagagcaccagcaccgcctacatggaactgagcagcctgagaagcgaggacaccgccgtgtactattgcgccagaggcaacggcaattacgccctggacgccatggattattggggccagggaaccctggtcaccgtttctagcggaggcggaggatctggtggcggaggaagtggcggaggcggttctgaaattgtgctgacacagagccccggcacactgtcactttctccaggcgaaagagccacactgagctgcagagccagccagtctgtgtccagcagctacttcgcctggtatcagcagaagccaggccaggctcctcggctgttgatctatggcgcctcttctagagccacaggcatccccgatagattcagcggctctggcagcggcaccgatttcaccctgacaatcagcagactggaacccgaggacttcgctgtgtactactgccagcagtactacgacagccccatcacctttggccagggcacaagactggaaatcaaa

SEQ ID NO: 31 - protein, 12 aa, Homo sapiens
  source 1..12: note = human IgG4 hinge domain
ESKYGPPCPSCP

SEQ ID NO: 32 - protein, 42 aa, Homo sapiens
  source 1..42: note = human CD8 hinge domain.
PAPRPPTPAPTIASQPLSLRPEACRPAAGGAVHTRGLDFACD

SEQ ID NO: 33 - protein, 21 aa, Homo sapiens
  source 1..21: note = transmembrane domain of human CD8
IYIWAPLAGTCGVLLLSLVIT

SEQ ID NO: 34 - protein, 27 aa, Homo sapiens
  source 1..27: note = transmembrane domain of human CD28
FWVLVVVGGVLACYSLLVTVAFIIFWV

SEQ ID NO: 35 - protein, 27 aa, Homo sapiens
  source 1..27: note = transmembrane domain of human CD137
IISFFLALTSTALLFLLFFLTLRFSVV

SEQ ID NO: 36 - protein, 42 aa, Homo sapiens
  source 1..42: note = intracellular signaling domain of human CD137
KRGRKKLLYIFKQPFMRPVQTTQEEDGCSCRFPEEEEGGCEL

SEQ ID NO: 37 - protein, 18 aa, Homo sapiens
  source 1..18: note = intracellular part of human CD8
LYCNHRNRRRVCKCPRVD

SEQ ID NO: 38 - protein, 8 aa, synthetic construct
  source 1..8: note = FLAG tag
DYKDDDDK

SEQ ID NO: 39 - skipped

SEQ ID NO: 40 - protein, 20 aa, Mus musculus
  source 1..20: note = murine kappa light chain leader sequence
METDTLLLWVLLLWVPGSTG

SEQ ID NO: 41 - protein, 318 aa, synthetic construct
  source 1..318: note = switch receptor (SR01)
QVQLVQSGAEVKKPGSSVKVSCKASGYTPSSNVISWVRQAPGQGLEWMGGVIPIVDIANYAQRFKGRVTITADESTSTTYMELSSLRSEDTAVYYCASTLGLVLDAMDYWGQGTLVTVSSGGGGSGGGGSGGGGSETVLTQSPGTLSLSPGERATLSCRASQSLGSSYLAWYQQKPGQAPRLLIYGASSRAPGIPDRFSGSGSGTDFTLTISRLEPEDFAVYYCQQYADSPITFGQGTRLEIKESKYGPPCPSCPIYIWAPLAGTCGVLLLSLVITKRGRKKLLYIFKQPFMRPVQTTQEEDGCSCRFPEEEEGGCEL

SEQ ID NO: 42 - protein, 336 aa, synthetic construct
  source 1..336: note = switch receptor (SR02)
QVQLVQSGAEVKKPGSSVKVSCKASGYTPSSNVISWVRQAPGQGLEWMGGVIPIVDIANYAQRFKGRVTITADESTSTTYMELSSLRSEDTAVYYCASTLGLVLDAMDYWGQGTLVTVSSGGGGSGGGGSGGGGSETVLTQSPGTLSLSPGERATLSCRASQSLGSSYLAWYQQKPGQAPRLLIYGASSRAPGIPDRFSGSGSGTDFTLTISRLEPEDFAVYYCQQYADSPITFGQGTRLEIKESKYGPPCPSCPIYIWAPLAGTCGVLLLSLVITLYCNHRNRRRVCKCPRVDKRGRKKLLYIFKQPFMRPVQTTQEEDGCSCRFPEEEEGGCEL

SEQ ID NO: 43 - protein, 366 aa, synthetic construct
  source 1..366: note = switch receptor (SR03)
QVQLVQSGAEVKKPGSSVKVSCKASGYTPSSNVISWVRQAPGQGLEWMGGVIPIVDIANYAQRFKGRVTITADESTSTTYMELSSLRSEDTAVYYCASTLGLVLDAMDYWGQGTLVTVSSGGGGSGGGGSGGGGSETVLTQSPGTLSLSPGERATLSCRASQSLGSSYLAWYQQKPGQAPRLLIYGASSRAPGIPDRFSGSGSGTDFTLTISRLEPEDFAVYYCQQYADSPITFGQGTRLEIKPAPRPPTPAPTIASQPLSLRPEACRPAAGGAVHTRGLDFACDIYIWAPLAGTCGVLLLSLVITLYCNHRNRRRVCKCPRVDKRGRKKLLYIFKQPFMRPVQTTQEEDGCSCRFPEEEEGGCEL

SEQ ID NO: 44 - protein, 324 aa, synthetic construct
  source 1..324: note = switch receptor (SR04)
QVQLVQSGAEVKKPGSSVKVSCKASGYTPSSNVISWVRQAPGQGLEWMGGVIPIVDIANYAQRFKGRVTITADESTSTTYMELSSLRSEDTAVYYCASTLGLVLDAMDYWGQGTLVTVSSGGGGSGGGGSGGGGSETVLTQSPGTLSLSPGERATLSCRASQSLGSSYLAWYQQKPGQAPRLLIYGASSRAPGIPDRFSGSGSGTDFTLTISRLEPEDFAVYYCQQYADSPITFGQGTRLEIKESKYGPPCPSCPFWVLVVVGGVLACYSLLVTVAFIIFWVKRGRKKLLYIFKQPFMRPVQTTQEEDGCSCRFPEEEEGGCEL

SEQ ID NO: 45 - protein, 318 aa, synthetic construct
  source 1..318: note = switch receptor (SR05)
QVQLVQSGAEVKKPGSSVKVSCKASGYTFSSNVISWVRQAPGQGLEWMGGVIPIVDIANYAQRFKGRVTITADESTSTTYMELSSLRSEDTAVYYCALPRAFVLDAMDYWGQGTLVTVSSGGGGSGGGGSGGGGSETVLTQSPGTLSLSPGERATLSCRASQSLGSSYLAWYQQKPGQAPRLLIYGASSRAPGIPDRFSGSGSGTDFTLTISRLEPEDFAVYYCQQYADSPITFGQGTRLEIKESKYGPPCPSCPIYIWAPLAGTCGVLLLSLVITKRGRKKLLYIFKQPFMRPVQTTQEEDGCSCRFPEEEEGGCEL

SEQ ID NO: 46 - protein, 336 aa, unidentified
  source 1..336: note = switch receptor (SR06)
QVQLVQSGAEVKKPGSSVKVSCKASGYTFSSNVISWVRQAPGQGLEWMGGVIPIVDIANYAQRFKGRVTITADESTSTTYMELSSLRSEDTAVYYCALPRAFVLDAMDYWGQGTLVTVSSGGGGSGGGGSGGGGSETVLTQSPGTLSLSPGERATLSCRASQSLGSSYLAWYQQKPGQAPRLLIYGASSRAPGIPDRFSGSGSGTDFTLTISRLEPEDFAVYYCQQYADSPITFGQGTRLEIKESKYGPPCPSCPIYIWAPLAGTCGVLLLSLVITLYCNHRNRRRVCKCPRVDKRGRKKLLYIFKQPFMRPVQTTQEEDGCSCRFPEEEEGGCEL

SEQ ID NO: 47 - protein, 366 aa, synthetic construct
  source 1..366: note = switch receptor (SR07)
QVQLVQSGAEVKKPGSSVKVSCKASGYTFSSNVISWVRQAPGQGLEWMGGVIPIVDIANYAQRFKGRVTITADESTSTTYMELSSLRSEDTAVYYCALPRAFVLDAMDYWGQGTLVTVSSGGGGSGGGGSGGGGSETVLTQSPGTLSLSPGERATLSCRASQSLGSSYLAWYQQKPGQAPRLLIYGASSRAPGIPDRFSGSGSGTDFTLTISRLEPEDFAVYYCQQYADSPITFGQGTRLEIKPAPRPPTPAPTIASQPLSLRPEACRPAAGGAVHTRGLDFACDIYIWAPLAGTCGVLLLSLVITLYCNHRNRRRVCKCPRVDKRGRKKLLYIFKQPFMRPVQTTQEEDGCSCRFPEEEEGGCEL

SEQ ID NO: 48 - protein, 324 aa, synthetic construct
  source 1..324: note = switch receptor (SR08)
QVQLVQSGAEVKKPGSSVKVSCKASGYTFSSNVISWVRQAPGQGLEWMGGVIPIVDIANYAQRFKGRVTITADESTSTTYMELSSLRSEDTAVYYCALPRAFVLDAMDYWGQGTLVTVSSGGGGSGGGGSGGGGSETVLTQSPGTLSLSPGERATLSCRASQSLGSSYLAWYQQKPGQAPRLLIYGASSRAPGIPDRFSGSGSGTDFTLTISRLEPEDFAVYYCQQYADSPITFGQGTRLEIKESKYGPPCPSCPFWVLVVVGGVLACYSLLVTVAFIIFWVKRGRKKLLYIFKQPFMRPVQTTQEEDGCSCRFPEEEEGGCEL

SEQ ID NO: 49 - protein, 319 aa, synthetic construct
  source 1..319: note = switch receptor (SR09)
QVQLVQSGAEVKKPGSSVKVSCKASGGTFSTSFINWVRQAPGQGLEWMGGIIPIFDITNYAQKFQSRVTITADKSTSTAYMELSSLRSEDTAVYYCARGNGNYALDAMDYWGQGTLVTVSSGGGGSGGGGSGGGGSEIVLTQSPGTLSLSPGERATLSCRASQSVSSSYFAWYQQKPGQAPRLLIYGASSRATGIPDRFSGSGSGTDFTLTISRLEPEDFAVYYCQQYYDSPITFGQGTRLEIKESKYGPPCPSCPIYIWAPLAGTCGVLLLSLVITKRGRKKLLYIFKQPFMRPVQTTQEEDGCSCRFPEEEEGGCEL

SEQ ID NO: 50 - protein, 337 aa, synthetic construct
  source 1..337: note = switch receptor (SR10)
QVQLVQSGAEVKKPGSSVKVSCKASGGTFSTSFINWVRQAPGQGLEWMGGIIPIFDITNYAQKFQSRVTITADKSTSTAYMELSSLRSEDTAVYYCARGNGNYALDAMDYWGQGTLVTVSSGGGGSGGGGSGGGGSEIVLTQSPGTLSLSPGERATLSCRASQSVSSSYFAWYQQKPGQAPRLLIYGASSRATGIPDRFSGSGSGTDFTLTISRLEPEDFAVYYCQQYYDSPITFGQGTRLEIKESKYGPPCPSCPIYIWAPLAGTCGVLLLSLVITLYCNHRNRRRVCKCPRVDKRGRKKLLYIFKQPFMRPVQTTQEEDGCSCRFPEEEEGGCEL

SEQ ID NO: 51 - protein, 367 aa, synthetic construct
  source 1..367: note = switch receptor (SR11)
QVQLVQSGAEVKKPGSSVKVSCKASGGTFSTSFINWVRQAPGQGLEWMGGIIPIFDITNYAQKFQSRVTITADKSTSTAYMELSSLRSEDTAVYYCARGNGNYALDAMDYWGQGTLVTVSSGGGGSGGGGSGGGGSEIVLTQSPGTLSLSPGERATLSCRASQSVSSSYFAWYQQKPGQAPRLLIYGASSRATGIPDRFSGSGSGTDFTLTISRLEPEDFAVYYCQQYYDSPITFGQGTRLEIKPAPRPPTPAPTIASQPLSLRPEACRPAAGGAVHTRGLDFACDIYIWAPLAGTCGVLLLSLVITLYCNHRNRRRVCKCPRVDKRGRKKLLYIFKQPFMRPVQTTQEEDGCSCRFPEEEEGGCEL

SEQ ID NO: 52 - protein, 325 aa, synthetic construct
  source 1..325: note = switch receptor (SR12)
QVQLVQSGAEVKKPGSSVKVSCKASGGTFSTSFINWVRQAPGQGLEWMGGIIPIFDITNYAQKFQSRVTITADKSTSTAYMELSSLRSEDTAVYYCARGNGNYALDAMDYWGQGTLVTVSSGGGGSGGGGSGGGGSEIVLTQSPGTLSLSPGERATLSCRASQSVSSSYFAWYQQKPGQAPRLLIYGASSRATGIPDRFSGSGSGTDFTLTISRLEPEDFAVYYCQQYYDSPITFGQGTRLEIKESKYGPPCPSCPFWVLVVVGGVLACYSLLVTVAFIIFWVKRGRKKLLYIFKQPFMRPVQTTQEEDGCSCRFPEEEEGGCEL

SEQ ID NO: 53 - protein, 324 aa, synthetic construct
  source 1..324: note = switch receptor (SR1-2)
QVQLVQSGAEVKKPGSSVKVSCKASGYTPSSNVISWVRQAPGQGLEWMGGVIPIVDIANYAQRFKGRVTITADESTSTTYMELSSLRSEDTAVYYCASTLGLVLDAMDYWGQGTLVTVSSGGGGSGGGGSGGGGSETVLTQSPGTLSLSPGERATLSCRASQSLGSSYLAWYQQKPGQAPRLLIYGASSRAPGIPDRFSGSGSGTDFTLTISRLEPEDFAVYYCQQYADSPITFGQGTRLEIKESKYGPPCPSCPIISFFLALTSTALLFLLFFLTLRFSVVKRGRKKLLYIFKQPFMRPVQTTQEEDGCSCRFPEEEEGGCEL

SEQ ID NO: 54 - protein, 324 aa, synthetic construct
  source 1..324: note = switch receptor (SR2-2)
QVQLVQSGAEVKKPGSSVKVSCKASGYTFSSNVISWVRQAPGQGLEWMGGVIPIVDIANYAQRFKGRVTITADESTSTTYMELSSLRSEDTAVYYCALPRAFVLDAMDYWGQGTLVTVSSGGGGSGGGGSGGGGSETVLTQSPGTLSLSPGERATLSCRASQSLGSSYLAWYQQKPGQAPRLLIYGASSRAPGIPDRFSGSGSGTDFTLTISRLEPEDFAVYYCQQYADSPITFGQGTRLEIKESKYGPPCPSCPIISFFLALTSTALLFLLFFLTLRFSVVKRGRKKLLYIFKQPFMRPVQTTQEEDGCSCRFPEEEEGGCEL

SEQ ID NO: 55 - protein, 325 aa, synthetic construct
  source 1..325: note = switch receptor (SR3-2)
QVQLVQSGAEVKKPGSSVKVSCKASGGTFSTSFINWVRQAPGQGLEWMGGIIPIFDITNYAQKFQSRVTITADKSTSTAYMELSSLRSEDTAVYYCARGNGNYALDAMDYWGQGTLVTVSSGGGGSGGGGSGGGGSEIVLTQSPGTLSLSPGERATLSCRASQSVSSSYFAWYQQKPGQAPRLLIYGASSRATGIPDRFSGSGSGTDFTLTISRLEPEDFAVYYCQQYYDSPITFGQGTRLEIKESKYGPPCPSCPIISFFLALTSTALLFLLFFLTLRFSVVKRGRKKLLYIFKQPFMRPVQTTQEEDGCSCRFPEEEEGGCEL

SEQ ID NO: 56 - DNA, 1008 bp, synthetic construct
  source 1..1008: mol_type = other DNA; note = nucleic acid encoding SR02
caggtgcagctggttcaatctggcgccgaagtgaagaaacccggcagctctgtgaaggtgtcctgcaaggccagcggctacacccctagcagcaatgtgatcagctgggtccgacaggcccctggacaaggacttgaatggatgggcggcgtgatccccatcgtggatatcgccaattacgcccagcggttcaagggcagagtgaccatcacagccgatgagagcaccagcaccacctacatggaactgagcagcctgagaagcgaggacaccgccgtgtactactgtgcctctacactgggccttgtgctggacgccatggattattggggccagggcacactggtcaccgtttctagcggaggcggaggatctggtggcggaggaagtggcggaggcggttctgaaacagtgctgacacagagccccggcacactgtctcttagccctggcgaaagagccacactgagctgtagagcctctcagagcctgggcagctcttacctggcttggtatcagcagaagcccggccaggctcctagactgctgatctatggcgcctcttctagagcccctggcatccccgatagattttctggcagcggctccggcaccgacttcaccctgacaatcagcagactggaacccgaggactttgccgtgtattattgccagcagtacgccgactctcccatcacctttggccagggaacacgcctggaaatcaaagagtctaagtacggccctccttgtcctagctgccccatctatatttgggcccctctggccggaacatgcggagtgttgctgctgagcctggtcatcaccctgtactgcaaccacagaaaccggcggagagtgtgcaagtgccccagagtggataagcggggcagaaagaagctgctgtacatcttcaagcagcccttcatgcggcccgtgcagaccacacaagaggaagatggctgctcctgcagattccccgaggaagaagaaggcggctgcgagctt